European Patent Specification EP 3 976 764 B1, published July 23, 2025. Title: METHODS FOR DETECTING A MYCOBACTERIUM TUBERCULOSIS INFECTION. Applicant: ViTi Incorporated Oregon Health & Science University Lewinsohn, Deborah A. Nyendak, Melissa Swarbrick, Gwendolyn Mooney, Jeffrey. The sequence listing filed with the application follows.

SEQUENCE LISTING (64 sequences)

SEQ ID NO: 1 - protein, 15 aa, Artificial sequence
  synthetic sequence
RPELPVRNYIRIPAL

SEQ ID NO: 2 - protein, 15 aa, Artificial sequence
  synthetic sequence
LHEARTAALNLFVVV

SEQ ID NO: 3 - protein, 15 aa, Artificial sequence
  synthetic sequence
WMGPASMAMVAAAQP

SEQ ID NO: 4 - protein, 11 aa, Artificial sequence
  synthetic sequence
GPRYGFKPTVM

SEQ ID NO: 5 - protein, 13 aa, Artificial sequence
  synthetic sequence
TLFEKLEPMASIL

SEQ ID NO: 6 - protein, 13 aa, Artificial sequence
  synthetic sequence
YQTYMYTGQYDGY

SEQ ID NO: 7 - protein, 16 aa, Artificial sequence
  synthetic sequence
IAPHFVRVRMVSPTLF

SEQ ID NO: 8 - protein, 12 aa, Artificial sequence
  synthetic sequence
YYLGEPIVQAVL

SEQ ID NO: 9 - protein, 11 aa, Artificial sequence
  synthetic sequence
QTVEDEARRMW

SEQ ID NO: 10 - protein, 16 aa, Artificial sequence
  synthetic sequence
AMSAQAFHQGESSAAF

SEQ ID NO: 11 - protein, 11 aa, Artificial sequence
  synthetic sequence
RRRCRPWLHRR

SEQ ID NO: 12 - protein, 12 aa, Artificial sequence
  synthetic sequence
TQALQALTIPSF

SEQ ID NO: 13 - protein, 13 aa, Artificial sequence
  synthetic sequence
RQFHHPLIYVLLV

SEQ ID NO: 14 - protein, 13 aa, Artificial sequence
  synthetic sequence
YVGLYLPFLDMSF

SEQ ID NO: 15 - protein, 9 aa, Artificial sequence
  synthetic sequence
NEIRALMAL

SEQ ID NO: 16 - protein, 15 aa, Artificial sequence
  synthetic sequence
SLLDAHIPQLVASQS

SEQ ID NO: 17 - protein, 15 aa, Artificial sequence
  synthetic sequence
LDAHIPQLVASQSAF

SEQ ID NO: 18 - protein, 16 aa, Artificial sequence
  synthetic sequence
HTIGQAEQAAMSAQAF

SEQ ID NO: 19 - protein, 15 aa, Artificial sequence
  synthetic sequence
AEQAAMSAQAFHQGE

SEQ ID NO: 20 - protein, 9 aa, Artificial sequence
  synthetic sequence
LESDPYHGL

SEQ ID NO: 21 - protein, 15 aa, Artificial sequence
  synthetic sequence
ARILRQFHHPLIYVL

SEQ ID NO: 22 - protein, 14 aa, Artificial sequence
  synthetic sequence
GLKEFVDAAVIFGV

SEQ ID NO: 23 - protein, 9 aa, Artificial sequence
  synthetic sequence
QESKAEAAL

SEQ ID NO: 24 - protein, 15 aa, Artificial sequence
  synthetic sequence
VAQYTPEQWWPFIGN

SEQ ID NO: 25 - protein, 14 aa, Artificial sequence
  synthetic sequence
TPEQWWPFIGNLSL

SEQ ID NO: 26 - protein, 12 aa, Artificial sequence
  synthetic sequence
AELQNGHDVVVF

SEQ ID NO: 27 - protein, 9 aa, Artificial sequence
  synthetic sequence
  misc_feature (1)..(9): Xaa can be any naturally occurring amino acid
XXXXXXXXX

SEQ ID NO: 28 - protein, 12 aa, Artificial sequence
  synthetic sequence
YAHNPQYPLNIL

SEQ ID NO: 29 - protein, 9 aa, Artificial sequence
  synthetic sequence
ILSDLNAFM

SEQ ID NO: 30 - protein, 11 aa, Artificial sequence
  synthetic sequence
TAAEVANAVPL

SEQ ID NO: 31 - protein, 11 aa, Artificial sequence
  synthetic sequence
AEAEPAAWLRF

SEQ ID NO: 32 - protein, 16 aa, Artificial sequence
  synthetic sequence
ATIAVMSLMGSSRFDV

SEQ ID NO: 33 - protein, 15 aa, Artificial sequence
  synthetic sequence
YQQLSRQMMTAFHDQ

SEQ ID NO: 34 - protein, 16 aa, Artificial sequence
  synthetic sequence
SRQMMTAFHDQFVQAL

SEQ ID NO: 35 - protein, 9 aa, Artificial sequence
  synthetic sequence
AEASAAQTM

SEQ ID NO: 36 - protein, 14 aa, Artificial sequence
  synthetic sequence
APARALLGHPLISA

SEQ ID NO: 37 - protein, 12 aa, Artificial sequence
  synthetic sequence
RRRWLGRQRRRR

SEQ ID NO: 38 - protein, 13 aa, Artificial sequence
  synthetic sequence
RRRRWCRWQRRCR

SEQ ID NO: 39 - protein, 15 aa, Artificial sequence
  synthetic sequence
RRQRWRWRCRQRRLR

SEQ ID NO: 40 - protein, 15 aa, Artificial sequence
  synthetic sequence
AAIAATEAQYAEMWA

SEQ ID NO: 41 - protein, 15 aa, Artificial sequence
  synthetic sequence
ATEAQYAEMWAQDAA

SEQ ID NO: 42 - protein, 13 aa, Artificial sequence
  synthetic sequence
AVSQATDPLSLLI

SEQ ID NO: 43 - protein, 13 aa, Artificial sequence
  synthetic sequence
LLIETVTQALQAL

SEQ ID NO: 44 - protein, 15 aa, Artificial sequence
  synthetic sequence
ASGVLPRYGVRLTVM

SEQ ID NO: 45 - protein, 13 aa, Artificial sequence
  synthetic sequence
GPMMAAGAAWNGL

SEQ ID NO: 46 - protein, 11 aa, Artificial sequence
  synthetic sequence
SVITRLTTESW

SEQ ID NO: 47 - protein, 15 aa, Artificial sequence
  synthetic sequence
ASMAMVAAAQPYLAW

SEQ ID NO: 48 - protein, 15 aa, Artificial sequence
  synthetic sequence
MDYFIRMWNQAALAM

SEQ ID NO: 49 - protein, 12 aa, Artificial sequence
  synthetic sequence
VYQAETAVNTLF

SEQ ID NO: 50 - protein, 15 aa, Artificial sequence
  synthetic sequence
LAAPPPQRAAMAAQL

SEQ ID NO: 51 - protein, 14 aa, Artificial sequence
  synthetic sequence
PPQRAAMAAQLQAV

SEQ ID NO: 52 - protein, 11 aa, Artificial sequence
  synthetic sequence
EQQEQASQQIL

SEQ ID NO: 53 - protein, 9 aa, Artificial sequence
  synthetic sequence
AFRNIVNML

SEQ ID NO: 54 - protein, 9 aa, Artificial sequence
  synthetic sequence
TMAQMNQAF

SEQ ID NO: 55 - protein, 15 aa, Artificial sequence
  synthetic sequence
VSTLLVASAWWLFAW

SEQ ID NO: 56 - protein, 9 aa, Artificial sequence
  synthetic sequence
WELDNGAGL

SEQ ID NO: 57 - protein, 15 aa, Artificial sequence
  synthetic sequence
AALNLFVVVEAFYLF

SEQ ID NO: 58 - protein, 11 aa, Artificial sequence
  synthetic sequence
GMMPGMASAAK

SEQ ID NO: 59 - protein, 11 aa, Artificial sequence
  synthetic sequence
MASAAKGTGAY

SEQ ID NO: 60 - protein, 15 aa, Artificial sequence
  synthetic sequence
YQQLSRQMMTAFHDQ

SEQ ID NO: 61 - protein, 16 aa, Artificial sequence
  synthetic sequence
SRQMMTAFHDQFVQAL

SEQ ID NO: 62 - protein, 15 aa, Artificial sequence
  synthetic sequence
FVGDYVTAGGLLGWC

SEQ ID NO: 63 - protein, 10 aa, Artificial sequence
  synthetic sequence
FIIDPTISAI

SEQ ID NO: 64 - protein, 15 aa, Artificial sequence
  synthetic sequence
NGFQLRRPLFPPLPG